European Patent Specification EP 4 251 749 B1, published August 7, 2024. Title: Cytidine deaminase variants for base editing. Applicant: CONSIGLIO NAZIONALE DELLE RICERCHE. The sequence listing filed with the application follows.

SEQUENCE LISTING (4 sequences)

SEQ ID NO: 1 - DNA, 690 bp, Homo sapiens
atgagttccgagacaggccctgtagctgttgatcccactctgaggagaagaattgagccccacgagtttgaagtcttctttgacccccgggaacttcggaaagagacctgtctgctgtatgagatcaactggggaggaaggcacagcatctggcgacacacgagccaaaacaccaacaaacacgttgaagtcaatttcatagaaaaatttactacagaaagatacttttgtccaaacaccagatgctccattacctggttcctgtcctggagtccctgtggggagtgctccagggccattacagaatttttgagccgatacccccatgtaactctgtttatttatatagcacggctttatcaccacgcagatcctcgaaatcggcaaggactcagggaccttattagcagcggtgttactatccagatcatgacggagcaagagtctggctactgctggaggaattttgtcaactactccccttcgaatgaagctcattggccaaggtacccccatctgtgggtgaggctgtacgtactggaactctactgcatcattttaggacttccaccctgtttaaatattttaagaagaaaacaacctcaactcacgtttttcacgattgctcttcaaagctgccattaccaaaggctaccaccccacatcctgtgggccacagggttgaaatga

SEQ ID NO: 2 - DNA, 687 bp, Synthetic
atgagttccgagacaggccctgtagctgttgatcccactctgaggagaagaattgagccccacgagtttgaagtcttctttgacccccgggaacttcggaaagagacctgtctgctgtatgagatcaactggggaggaaggcacagcatctggcgacacacgagccaaaacaccaacaaacacgttgaagtcaatctcatagaaaaatttactacagaaagatacttttgtccaaacaccagatgctccattacctggttcctgtcctggagtccctgtggggagtgctccagggccattacagaatttttgagccgatacccccatgtaactctgtttatttatatagcacggctttatcaccacgcagatcctcgaaatcggcaaggactcagggaccttattagcagcggtgttactatccagatcatgacggagcaagagtctggctactgctggaggaattttgtcaactactccccctcgaatgaagctcattggccaaggtacccccatctgtgggtgaggctgtacatactggaactctactgcatcattttaggacttccaccctgtttaaatattttaagaagaaaacaacctcaactcacgtttttcacgattgctcttcaaagctgccattaccaaaggctaccaccccacatcctgtgggccacagggttgaaa

SEQ ID NO: 3 - DNA, 687 bp, Synthetic
atgagttccgagacaggccctgtagctgttgatcccactctgaggagaagaattgagccccacgagtttgaagtcttctttgacccccgggaacttcggaaagagacctgtctgctgtatgagatcaactggggaggaaggcacagcatctggcgacacacgagccaaaacaccaacaaacacgttgaagtcaatttcatagaaaaatttactacagaaagatacttttgtccaaacaccagatgctccattacctggttcctgtcctggagtccctgtggggagtgctccagggccattacagaatttttgagccgatacccccatgtaactctgtttatttatatagcacggctttatcaccacgcagatcctcgaaatcggcaaggactcagggaccttattagcagcggtgttactatccagatcatgacggagcaagagtctggctactgctggaggaattttgtcaactactccccttcgaatgaagctcattggccaaggtacccccatctgtgggtgaggctgtacgtactggaactctactgcatcattttaggacttccaccctgtttaaataatttaagaagaaaacaacctcaactcacgtttttcacgattgctcttcaaagctgccattaccaaaggctaccaccccacatcctgtgggccacagggttgaaa

SEQ ID NO: 4 - DNA, 690 bp, Synthetic
atgagttccgagacaggccctgtagctgttgatcccactctgaggagaagaattgagccccacgagtttgaagtcttctttgacccccgggaacttcggaaagagacctgtctgctgtatgagatcaactggggaggaaggcacagcatctggcgacacacgagccaaaacaccaacaaacacgttgaagtcaatttcatagaaaaatttactacagaaagatacttttgtccaaacaccagacgctccattacctggttcctgtcctggagtccctgtggggagtgctccagggccattacagaatttttgagccgatacccccatgtaactctgtttatttatatagcacggctttatcaccacgcagatcctcgaaatcggcaaggactcagggaccttattagcagcggtgttactatccagatcatgacggagcaagagtctggctactgctggaggaattttgtcaactactccccttcgaatgaagctcattggccaaggtacccccatctgtgggtgaggctgtacgtactggaactctactgcatcattttaggacttccaccctgtttaaatattttaagaagaaaacaacctcaactcacgtttttcacgattgctcttcaaagctgccattaccaaaggctaccaccccacatcctgtgggccacagggttgaaatgt